European Patent Specification EP 4 087 931 B1, published December 25, 2024. Title: Novel TLR9 Agonists. Applicant: SBI Biotech Co., Ltd. The sequence listing filed with the application follows.

SEQUENCE LISTING (63 sequences)

SEQ ID NO: 1 - DNA, 11 bp, Artificial Sequence
  common sequence motif
tcgcaacgttt

SEQ ID NO: 2 - DNA, 24 bp, Artificial Sequence
  common sequence motif
  misc_feature (12)..(12): n stands for any base
  misc_feature (18)..(18): n stands for any base
  misc_feature (21)..(21): n stands for any base
  misc_feature (22)..(22): n stands for any base
tcgcaacgtttncgacgncgnncg

SEQ ID NO: 3 - DNA, 24 bp, Artificial Sequence
  common sequence motif
tcgcaacgtttrcgacgkcgbdcg

SEQ ID NO: 4 - DNA, 25 bp, Artificial Sequence
  common sequence motif
  misc_feature (22)..(22): n stands for any base
tcgcaacgtttrcgacgkcgbncgr

SEQ ID NO: 5 - DNA, 24 bp, Artificial Sequence
  common partially phosphorothioated stretch
  misc_feature (12)..(12): n stands for any base
  misc_feature (18)..(18): n stands for any base
  misc_feature (21)..(21): n stands for any base
  misc_feature (22)..(22): n stands for any base
  modified_base (1)..(1): phosphorothioate-modified at 3' internucleotide bond
  modified_base (3)..(3): phosphorothioate-modified at 3' internucleotide bond
  modified_base (5)..(6): phosphorothioate-modified at 3' internucleotide bond
  modified_base (8)..(18): phosphorothioate-modified at 3' internucleotide bond
  modified_base (20)..(22): phosphorothioate-modified at 3' internucleotide bond
tcgcaacgtttncgacgncgnncg

SEQ ID NO: 6 - DNA, 25 bp, Artificial Sequence
  A001
  modified_base (1)..(24): phosphorothioate-modified at 3' internucleotide bond
tcgcaacgtttgcgacgtcggtcga

SEQ ID NO: 7 - DNA, 25 bp, Artificial Sequence
  A002
  modified_base (1)..(24): phosphorothioate-modified at 3' internucleotide bond
tcgcaacgtttgcgacggcgctcga

SEQ ID NO: 8 - DNA, 25 bp, Artificial Sequence
  A003
  modified_base (1)..(24): phosphorothioate-modified at 3' internucleotide bond
tcgcaacgtttgcgacgtcgttcga

SEQ ID NO: 9 - DNA, 25 bp, Artificial Sequence
  A004
  modified_base (1)..(24): phosphorothioate-modified at 3' internucleotide bond
tcgcaacgtttgcgacggcgttcga

SEQ ID NO: 10 - DNA, 24 bp, Artificial Sequence
  A003#delA
  modified_base (1)..(23): phosphorothioate-modified at 3' internucleotide bond
tcgcaacgtttgcgacgtcgttcg

SEQ ID NO: 11 - DNA, 25 bp, Artificial Sequence
  A003#endG
  modified_base (1)..(24): phosphorothioate-modified at 3' internucleotide bond
tcgcaacgtttgcgacgtcgttcgg

SEQ ID NO: 12 - DNA, 25 bp, Artificial Sequence
  A011
  modified_base (1)..(24): phosphorothioate-modified at 3' internucleotide bond
tcgcaacgtttacgacgtcggtcga

SEQ ID NO: 13 - DNA, 25 bp, Artificial Sequence
  A012
  modified_base (1)..(24): phosphorothioate-modified at 3' internucleotide bond
tcgcaacgtttacgacggcgctcga

SEQ ID NO: 14 - DNA, 25 bp, Artificial Sequence
  A013
  modified_base (1)..(24): phosphorothioate-modified at 3' internucleotide bond
tcgcaacgtttacgacgtcgttcga

SEQ ID NO: 15 - DNA, 25 bp, Artificial Sequence
  A014
  modified_base (1)..(24): phosphorothioate-modified at 3' internucleotide bond
tcgcaacgtttacgacggcgttcga

SEQ ID NO: 16 - DNA, 25 bp, Artificial Sequence
  A103
  modified_base (1)..(1): phosphorothioate-modified at 3' internucleotide bond
  modified_base (3)..(24): phosphorothioate-modified at 3' internucleotide bond
tcgcaacgtttgcgacgtcgttcga

SEQ ID NO: 17 - DNA, 25 bp, Artificial Sequence
  A203
  modified_base (1)..(1): phosphorothioate-modified at 3' internucleotide bond
  modified_base (3)..(6): phosphorothioate-modified at 3' internucleotide bond
  modified_base (8)..(24): phosphorothioate-modified at 3' internucleotide bond
tcgcaacgtttgcgacgtcgttcga

SEQ ID NO: 18 - DNA, 25 bp, Artificial Sequence
  A303
  modified_base (1)..(1): phosphorothioate-modified at 3' internucleotide bond
  modified_base (3)..(3): phosphorothioate-modified at 3' internucleotide bond
  modified_base (5)..(6): phosphorothioate-modified at 3' internucleotide bond
  modified_base (8)..(24): phosphorothioate-modified at 3' internucleotide bond
tcgcaacgtttgcgacgtcgttcga

SEQ ID NO: 19 - DNA, 25 bp, Artificial Sequence
  A403
  modified_base (1)..(1): phosphorothioate-modified at 3' internucleotide bond
  modified_base (3)..(3): phosphorothioate-modified at 3' internucleotide bond
  modified_base (5)..(12): phosphorothioate-modified at 3' internucleotide bond
  modified_base (14)..(15): phosphorothioate-modified at 3' internucleotide bond
  modified_base (17)..(24): phosphorothioate-modified at 3' internucleotide bond
tcgcaacgtttgcgacgtcgttcga

SEQ ID NO: 20 - DNA, 25 bp, Artificial Sequence
  A503
  modified_base (1)..(1): phosphorothioate-modified at 3' internucleotide bond
  modified_base (3)..(3): phosphorothioate-modified at 3' internucleotide bond
  modified_base (5)..(12): phosphorothioate-modified at 3' internucleotide bond
  modified_base (14)..(15): phosphorothioate-modified at 3' internucleotide bond
  modified_base (17)..(22): phosphorothioate-modified at 3' internucleotide bond
  modified_base (24)..(24): phosphorothioate-modified at 3' internucleotide bond
tcgcaacgtttgcgacgtcgttcga

SEQ ID NO: 21 - DNA, 25 bp, Artificial Sequence
  A603
  modified_base (1)..(1): phosphorothioate-modified at 3' internucleotide bond
  modified_base (3)..(3): phosphorothioate-modified at 3' internucleotide bond
  modified_base (5)..(6): phosphorothioate-modified at 3' internucleotide bond
  modified_base (8)..(18): phosphorothioate-modified at 3' internucleotide bond
  modified_base (20)..(22): phosphorothioate-modified at 3' internucleotide bond
  modified_base (24)..(24): phosphorothioate-modified at 3' internucleotide bond
tcgcaacgtttgcgacgtcgttcga

SEQ ID NO: 22 - DNA, 25 bp, Artificial Sequence
  A703
  modified_base (1)..(1): phosphorothioate-modified at 3' internucleotide bond
  modified_base (3)..(3): phosphorothioate-modified at 3' internucleotide bond
  modified_base (5)..(6): phosphorothioate-modified at 3' internucleotide bond
  modified_base (8)..(12): phosphorothioate-modified at 3' internucleotide bond
  modified_base (14)..(15): phosphorothioate-modified at 3' internucleotide bond
  modified_base (17)..(18): phosphorothioate-modified at 3' internucleotide bond
  modified_base (20)..(22): phosphorothioate-modified at 3' internucleotide bond
  modified_base (24)..(24): phosphorothioate-modified at 3' internucleotide bond
tcgcaacgtttgcgacgtcgttcga

SEQ ID NO: 23 - DNA, 25 bp, Artificial Sequence
  A601
  modified_base (1)..(1): phosphorothioate-modified at 3' internucleotide bond
  modified_base (3)..(3): phosphorothioate-modified at 3' internucleotide bond
  modified_base (5)..(6): phosphorothioate-modified at 3' internucleotide bond
  modified_base (8)..(18): phosphorothioate-modified at 3' internucleotide bond
  modified_base (20)..(22): phosphorothioate-modified at 3' internucleotide bond
  modified_base (24)..(24): phosphorothioate-modified at 3' internucleotide bond
tcgcaacgtttgcgacgtcggtcga

SEQ ID NO: 24 - DNA, 25 bp, Artificial Sequence
  A602
  modified_base (1)..(1): phosphorothioate-modified at 3' internucleotide bond
  modified_base (3)..(3): phosphorothioate-modified at 3' internucleotide bond
  modified_base (5)..(6): phosphorothioate-modified at 3' internucleotide bond
  modified_base (8)..(18): phosphorothioate-modified at 3' internucleotide bond
  modified_base (20)..(22): phosphorothioate-modified at 3' internucleotide bond
  modified_base (24)..(24): phosphorothioate-modified at 3' internucleotide bond
tcgcaacgtttgcgacggcgctcga

SEQ ID NO: 25 - skipped

SEQ ID NO: 26 - DNA, 25 bp, Artificial Sequence
  A604
  modified_base (1)..(1): phosphorothioate-modified at 3' internucleotide bond
  modified_base (3)..(3): phosphorothioate-modified at 3' internucleotide bond
  modified_base (5)..(6): phosphorothioate-modified at 3' internucleotide bond
  modified_base (8)..(18): phosphorothioate-modified at 3' internucleotide bond
  modified_base (20)..(22): phosphorothioate-modified at 3' internucleotide bond
  modified_base (24)..(24): phosphorothioate-modified at 3' internucleotide bond
tcgcaacgtttgcgacggcgttcga

SEQ ID NO: 27 - DNA, 25 bp, Artificial Sequence
  A605
  modified_base (1)..(1): phosphorothioate-modified at 3' internucleotide bond
  modified_base (3)..(3): phosphorothioate-modified at 3' internucleotide bond
  modified_base (5)..(6): phosphorothioate-modified at 3' internucleotide bond
  modified_base (8)..(18): phosphorothioate-modified at 3' internucleotide bond
  modified_base (20)..(22): phosphorothioate-modified at 3' internucleotide bond
  modified_base (24)..(24): phosphorothioate-modified at 3' internucleotide bond
tcgcaacgtttgcgacgccgttcga

SEQ ID NO: 28 - DNA, 25 bp, Artificial Sequence
  A606
  modified_base (1)..(1): phosphorothioate-modified at 3' internucleotide bond
  modified_base (3)..(3): phosphorothioate-modified at 3' internucleotide bond
  modified_base (5)..(6): phosphorothioate-modified at 3' internucleotide bond
  modified_base (8)..(18): phosphorothioate-modified at 3' internucleotide bond
  modified_base (20)..(22): phosphorothioate-modified at 3' internucleotide bond
  modified_base (24)..(24): phosphorothioate-modified at 3' internucleotide bond
tcgcaacgtttgcgacggcgtacga

SEQ ID NO: 29 - DNA, 25 bp, Artificial Sequence
  A607
  modified_base (1)..(1): phosphorothioate-modified at 3' internucleotide bond
  modified_base (3)..(3): phosphorothioate-modified at 3' internucleotide bond
  modified_base (5)..(6): phosphorothioate-modified at 3' internucleotide bond
  modified_base (8)..(18): phosphorothioate-modified at 3' internucleotide bond
  modified_base (20)..(22): phosphorothioate-modified at 3' internucleotide bond
  modified_base (24)..(24): phosphorothioate-modified at 3' internucleotide bond
tcgcaacgtttgcgacggcgtgcga

SEQ ID NO: 30 - DNA, 25 bp, Artificial Sequence
  A611
  modified_base (1)..(1): phosphorothioate-modified at 3' internucleotide bond
  modified_base (3)..(3): phosphorothioate-modified at 3' internucleotide bond
  modified_base (5)..(6): phosphorothioate-modified at 3' internucleotide bond
  modified_base (8)..(18): phosphorothioate-modified at 3' internucleotide bond
  modified_base (20)..(22): phosphorothioate-modified at 3' internucleotide bond
  modified_base (24)..(24): phosphorothioate-modified at 3' internucleotide bond
tcgcaacgtttacgacgtcggtcga

SEQ ID NO: 31 - DNA, 25 bp, Artificial Sequence
  A612
  modified_base (1)..(1): phosphorothioate-modified at 3' internucleotide bond
  modified_base (3)..(3): phosphorothioate-modified at 3' internucleotide bond
  modified_base (5)..(6): phosphorothioate-modified at 3' internucleotide bond
  modified_base (8)..(18): phosphorothioate-modified at 3' internucleotide bond
  modified_base (20)..(22): phosphorothioate-modified at 3' internucleotide bond
  modified_base (24)..(24): phosphorothioate-modified at 3' internucleotide bond
tcgcaacgtttacgacggcgctcga

SEQ ID NO: 32 - DNA, 25 bp, Artificial Sequence
  A613
  modified_base (1)..(1): phosphorothioate-modified at 3' internucleotide bond
  modified_base (3)..(3): phosphorothioate-modified at 3' internucleotide bond
  modified_base (5)..(6): phosphorothioate-modified at 3' internucleotide bond
  modified_base (8)..(18): phosphorothioate-modified at 3' internucleotide bond
  modified_base (20)..(22): phosphorothioate-modified at 3' internucleotide bond
  modified_base (24)..(24): phosphorothioate-modified at 3' internucleotide bond
tcgcaacgtttacgacgtcgttcga

SEQ ID NO: 33 - DNA, 25 bp, Artificial Sequence
  A601G
  modified_base (1)..(1): phosphorothioate-modified at 3' internucleotide bond
  modified_base (3)..(3): phosphorothioate-modified at 3' internucleotide bond
  modified_base (5)..(6): phosphorothioate-modified at 3' internucleotide bond
  modified_base (8)..(11): phosphorothioate-modified at 3' internucleotide bond
  modified_base (13)..(18): phosphorothioate-modified at 3' internucleotide bond
  modified_base (20)..(22): phosphorothioate-modified at 3' internucleotide bond
  modified_base (24)..(24): phosphorothioate-modified at 3' internucleotide bond
tcgcaacgtttgcgacgtcggtcga

SEQ ID NO: 34 - DNA, 25 bp, Artificial Sequence
  A611A
  modified_base (1)..(1): phosphorothioate-modified at 3' internucleotide bond
  modified_base (3)..(3): phosphorothioate-modified at 3' internucleotide bond
  modified_base (5)..(6): phosphorothioate-modified at 3' internucleotide bond
  modified_base (8)..(11): phosphorothioate-modified at 3' internucleotide bond
  modified_base (13)..(18): phosphorothioate-modified at 3' internucleotide bond
  modified_base (20)..(22): phosphorothioate-modified at 3' internucleotide bond
  modified_base (24)..(24): phosphorothioate-modified at 3' internucleotide bond
tcgcaacgtttacgacgtcggtcga

SEQ ID NO: 35 - DNA, 25 bp, Artificial Sequence
  A602G
  modified_base (1)..(1): phosphorothioate-modified at 3' internucleotide bond
  modified_base (3)..(3): phosphorothioate-modified at 3' internucleotide bond
  modified_base (5)..(6): phosphorothioate-modified at 3' internucleotide bond
  modified_base (8)..(11): phosphorothioate-modified at 3' internucleotide bond
  modified_base (13)..(18): phosphorothioate-modified at 3' internucleotide bond
  modified_base (20)..(22): phosphorothioate-modified at 3' internucleotide bond
  modified_base (24)..(24): phosphorothioate-modified at 3' internucleotide bond
tcgcaacgtttgcgacggcgctcga

SEQ ID NO: 36 - DNA, 25 bp, Artificial Sequence
  A612A
  modified_base (1)..(1): phosphorothioate-modified at 3' internucleotide bond
  modified_base (3)..(3): phosphorothioate-modified at 3' internucleotide bond
  modified_base (5)..(6): phosphorothioate-modified at 3' internucleotide bond
  modified_base (8)..(11): phosphorothioate-modified at 3' internucleotide bond
  modified_base (13)..(18): phosphorothioate-modified at 3' internucleotide bond
  modified_base (20)..(22): phosphorothioate-modified at 3' internucleotide bond
  modified_base (24)..(24): phosphorothioate-modified at 3' internucleotide bond
tcgcaacgtttacgacggcgctcga

SEQ ID NO: 37 - DNA, 25 bp, Artificial Sequence
  A603G?
  modified_base (1)..(1): phosphorothioate-modified at 3' internucleotide bond
  modified_base (3)..(3): phosphorothioate-modified at 3' internucleotide bond
  modified_base (5)..(6): phosphorothioate-modified at 3' internucleotide bond
  modified_base (8)..(11): phosphorothioate-modified at 3' internucleotide bond
  modified_base (13)..(18): phosphorothioate-modified at 3' internucleotide bond
  modified_base (20)..(22): phosphorothioate-modified at 3' internucleotide bond
  modified_base (24)..(24): phosphorothioate-modified at 3' internucleotide bond
tcgcaacgtttgcgacgtcgttcga

SEQ ID NO: 38 - DNA, 25 bp, Artificial Sequence
  A613A
  modified_base (1)..(1): phosphorothioate-modified at 3' internucleotide bond
  modified_base (3)..(3): phosphorothioate-modified at 3' internucleotide bond
  modified_base (5)..(6): phosphorothioate-modified at 3' internucleotide bond
  modified_base (8)..(11): phosphorothioate-modified at 3' internucleotide bond
  modified_base (13)..(18): phosphorothioate-modified at 3' internucleotide bond
  modified_base (20)..(22): phosphorothioate-modified at 3' internucleotide bond
  modified_base (24)..(24): phosphorothioate-modified at 3' internucleotide bond
tcgcaacgtttacgacgtcgttcga

SEQ ID NO: 39 - DNA, 25 bp, Artificial Sequence
  A601GendG
  modified_base (1)..(1): phosphorothioate-modified at 3' internucleotide bond
  modified_base (3)..(3): phosphorothioate-modified at 3' internucleotide bond
  modified_base (5)..(6): phosphorothioate-modified at 3' internucleotide bond
  modified_base (8)..(11): phosphorothioate-modified at 3' internucleotide bond
  modified_base (13)..(18): phosphorothioate-modified at 3' internucleotide bond
  modified_base (20)..(22): phosphorothioate-modified at 3' internucleotide bond
  modified_base (24)..(24): phosphorothioate-modified at 3' internucleotide bond
tcgcaacgtttgcgacgtcggtcgg

SEQ ID NO: 40 - DNA, 25 bp, Artificial Sequence
  A611AendG
  modified_base (1)..(1): phosphorothioate-modified at 3' internucleotide bond
  modified_base (3)..(3): phosphorothioate-modified at 3' internucleotide bond
  modified_base (5)..(6): phosphorothioate-modified at 3' internucleotide bond
  modified_base (8)..(11): phosphorothioate-modified at 3' internucleotide bond
  modified_base (13)..(18): phosphorothioate-modified at 3' internucleotide bond
  modified_base (20)..(22): phosphorothioate-modified at 3' internucleotide bond
  modified_base (24)..(24): phosphorothioate-modified at 3' internucleotide bond
tcgcaacgtttacgacgtcggtcgg

SEQ ID NO: 41 - DNA, 25 bp, Artificial Sequence
  A602GendG
  modified_base (1)..(1): phosphorothioate-modified at 3' internucleotide bond
  modified_base (3)..(3): phosphorothioate-modified at 3' internucleotide bond
  modified_base (5)..(6): phosphorothioate-modified at 3' internucleotide bond
  modified_base (8)..(11): phosphorothioate-modified at 3' internucleotide bond
  modified_base (13)..(18): phosphorothioate-modified at 3' internucleotide bond
  modified_base (20)..(22): phosphorothioate-modified at 3' internucleotide bond
  modified_base (24)..(24): phosphorothioate-modified at 3' internucleotide bond
tcgcaacgtttgcgacggcgctcgg

SEQ ID NO: 42 - DNA, 25 bp, Artificial Sequence
  A612AendG
  modified_base (1)..(1): phosphorothioate-modified at 3' internucleotide bond
  modified_base (3)..(3): phosphorothioate-modified at 3' internucleotide bond
  modified_base (5)..(6): phosphorothioate-modified at 3' internucleotide bond
  modified_base (8)..(11): phosphorothioate-modified at 3' internucleotide bond
  modified_base (13)..(18): phosphorothioate-modified at 3' internucleotide bond
  modified_base (20)..(22): phosphorothioate-modified at 3' internucleotide bond
  modified_base (24)..(24): phosphorothioate-modified at 3' internucleotide bond
tcgcaacgtttacgacggcgctcgg

SEQ ID NO: 43 - DNA, 25 bp, Artificial Sequence
  A603GendG
  modified_base (1)..(1): phosphorothioate-modified at 3' internucleotide bond
  modified_base (3)..(3): phosphorothioate-modified at 3' internucleotide bond
  modified_base (5)..(6): phosphorothioate-modified at 3' internucleotide bond
  modified_base (8)..(11): phosphorothioate-modified at 3' internucleotide bond
  modified_base (13)..(18): phosphorothioate-modified at 3' internucleotide bond
  modified_base (20)..(22): phosphorothioate-modified at 3' internucleotide bond
  modified_base (24)..(24): phosphorothioate-modified at 3' internucleotide bond
tcgcaacgtttgcgacgtcgttcgg

SEQ ID NO: 44 - DNA, 25 bp, Artificial Sequence
  A613AendG
  modified_base (1)..(1): phosphorothioate-modified at 3' internucleotide bond
  modified_base (3)..(3): phosphorothioate-modified at 3' internucleotide bond
  modified_base (5)..(6): phosphorothioate-modified at 3' internucleotide bond
  modified_base (8)..(11): phosphorothioate-modified at 3' internucleotide bond
  modified_base (13)..(18): phosphorothioate-modified at 3' internucleotide bond
  modified_base (20)..(22): phosphorothioate-modified at 3' internucleotide bond
  modified_base (24)..(24): phosphorothioate-modified at 3' internucleotide bond
tcgcaacgtttacgacgtcgttcgg

SEQ ID NO: 45 - DNA, 22 bp, Artificial Sequence
  CpG2395
  modified_base (1)..(21): phosphorothioate-modified at 3' internucleotide bond
tcgtcgttttcggcgcgcgccg

SEQ ID NO: 46 - DNA, 21 bp, Artificial Sequence
  CpG685
  modified_base (1)..(20): phosphorothioate-modified at 3' internucleotide bond
tcgtcgacgtcgttcgttctc

SEQ ID NO: 47 - DNA, 25 bp, Artificial Sequence
  M362
  modified_base (1)..(24): phosphorothioate-modified at 3' internucleotide bond
tcgtcgtcgttcgaacgacgttgat

SEQ ID NO: 48 - DNA, 30 bp, Artificial Sequence
  D60-1
  modified_base (1)..(29): phosphorothioate-modified at 3' internucleotide bond
tcgaacgttcgaacgttcgaacgttcgaat

SEQ ID NO: 49 - DNA, 18 bp, Artificial Sequence
  DV093
  modified_base (1)..(1): phosphorothioate-modified at 3' internucleotide bond
  modified_base (3)..(17): phosphorothioate-modified at 3' internucleotide bond
tcgtgcatcgatgcaacg

SEQ ID NO: 50 - DNA, 18 bp, Artificial Sequence
  DV093C
  modified_base (1)..(1): phosphorothioate-modified at 3' internucleotide bond
  modified_base (3)..(13): phosphorothioate-modified at 3' internucleotide bond
  modified_base (15)..(16): phosphorothioate-modified at 3' internucleotide bond
tcgtgcatcgatgcaacg

SEQ ID NO: 51 - DNA, 18 bp, Artificial Sequence
  DV094
  modified_base (1)..(17): phosphorothioate-modified at 3' internucleotide bond
aacaacaacgttgttgtt

SEQ ID NO: 52 - DNA, 18 bp, Artificial Sequence
  DV094C
  modified_base (1)..(2): phosphorothioate-modified at 3' internucleotide bond
  modified_base (4)..(5): phosphorothioate-modified at 3' internucleotide bond
  modified_base (7)..(8): phosphorothioate-modified at 3' internucleotide bond
  modified_base (10)..(17): phosphorothioate-modified at 3' internucleotide bond
aacaacaacgttgttgtt

SEQ ID NO: 53 - DNA, 24 bp, Artificial Sequence
  CpG2006
  modified_base (1)..(23): phosphorothioate-modified at 3' internucleotide bond
tcgtcgttttgtcgttttgtcgtt

SEQ ID NO: 54 - DNA, 25 bp, Artificial Sequence
  A sequence of the invention
tcgcaacgtttgcgacgtcggtcga

SEQ ID NO: 55 - DNA, 25 bp, Artificial Sequence
  A sequence of the invention
tcgcaacgtttgcgacggcgctcga

SEQ ID NO: 56 - DNA, 25 bp, Artificial Sequence
  A sequence of the invention
tcgcaacgtttgcgacgtcgttcga

SEQ ID NO: 57 - DNA, 25 bp, Artificial Sequence
  A sequence of the invention
tcgcaacgtttgcgacggcgttcga

SEQ ID NO: 58 - DNA, 24 bp, Artificial Sequence
  A sequence of the invention
tcgcaacgtttgcgacgtcgttcg

SEQ ID NO: 59 - DNA, 25 bp, Artificial Sequence
  A sequence of the invention
tcgcaacgtttgcgacgtcgttcgg

SEQ ID NO: 60 - DNA, 25 bp, Artificial Sequence
  A sequence of the invention
tcgcaacgtttacgacgtcggtcga

SEQ ID NO: 61 - DNA, 25 bp, Artificial Sequence
  A sequence of the invention
tcgcaacgtttacgacggcgctcga

SEQ ID NO: 62 - DNA, 25 bp, Artificial Sequence
  A sequence of the invention
tcgcaacgtttacgacgtcgttcga

SEQ ID NO: 63 - DNA, 25 bp, Artificial Sequence
  A sequence of the invention
tcgcaacgtttacgacggcgttcga